European Patent Application EP 4 321 168 A2, published February 14, 2024. Title: ENVIRONMENTALLY SENSITIVE COMPOSITIONS. Applicant: University of Rhode Island Board of Trustees. Application EP. The sequence listing filed with the application follows.

SEQUENCE LISTING (312 sequences)

SEQ ID NO: 1 - protein, 39 aa, unidentified
  REGION 1..39: note = Description of Unknown: pH-sensitive membrane polypeptide
AAEQNPIYWWARYADWLFTTPLLLLDLALLVDADEGTCG

SEQ ID NO: 2 - protein, 35 aa, unidentified
  REGION 1..35: note = Description of Unknown: Wild-type pH-sensitive membrane polypeptide
AEQNPIYWARYADWLFTTPLLLLDLALLVDADEGT

SEQ ID NO: 3 - protein, 36 aa, unidentified
  REGION 1..36: note = Description of Unknown: Wild-type pH-sensitive membrane polypeptide
GGEQNPIYWARYADWLFTTPLLLLDLALLVDADEGT

SEQ ID NO: 4 - protein, 35 aa, unidentified; identical to SEQ ID NO: 2
  REGION 1..35: note = Description of Unknown: Wild-type pH-sensitive membrane polypeptide

SEQ ID NO: 5 - protein, 38 aa, synthetic construct
  REGION 1..38: note = Description of Artificial Sequence: Synthetic polypeptide
AAEQNPIYWARYADWLFTTPLLLLDLALLVDADEGTCG

SEQ ID NO: 6 - protein, 38 aa, synthetic construct
  REGION 1..38: note = Description of Artificial Sequence: Synthetic polypeptide
GGEQNPIYWARYADWLFTTPLLLLDLALLVDADEGTCG

SEQ ID NO: 7 - protein, 37 aa, synthetic construct
  REGION 1..37: note = Description of Artificial Sequence: Synthetic polypeptide
ACEQNPIYWARYADWLFTTPLLLLDLALLVDADEGTG

SEQ ID NO: 8 - protein, 36 aa, synthetic construct
  REGION 1..36: note = Description of Artificial Sequence: Synthetic polypeptide
ACEQNPIYWARYADWLFTTPLLLLDLALLVDADEGT

SEQ ID NO: 9 - protein, 36 aa, synthetic construct
  REGION 1..36: note = Description of Artificial Sequence: Synthetic polypeptide
AKEQNPIYWARYADWLFTTPLLLLDLALLVDADEGT

SEQ ID NO: 10 - protein, 39 aa, synthetic construct
  REGION 1..39: note = Description of Artificial Sequence: Synthetic polypeptide
AAEQNPIYWARYADWLFTTPLLLLDLALLVDADEGTKCG

SEQ ID NO: 11 - protein, 36 aa, synthetic construct
  REGION 1..36: note = Description of Artificial Sequence: Synthetic polypeptide
AKEQNPIYWARYADWLFTTPLLLLDLALLVDADECT

SEQ ID NO: 12 - protein, 37 aa, synthetic construct
  REGION 1..37: note = Description of Artificial Sequence: Synthetic polypeptide
ACEQNPIYWARYANWLFTTPLLLLNLALLVDADEGTG

SEQ ID NO: 13 - protein, 37 aa, synthetic construct
  REGION 1..37: note = Description of Artificial Sequence: Synthetic polypeptide
ACEQNPIYWARYAKWLFTTPLLLLKLALLVDADEGTG

SEQ ID NO: 14 - protein, 36 aa, synthetic construct
  REGION 1..36: note = Description of Artificial Sequence: Synthetic polypeptide
GGEQNPIYWARYADWLFTTPLLLLDLALLVNANQGT

SEQ ID NO: 15 - protein, 36 aa, synthetic construct
  REGION 1..36: note = Description of Artificial Sequence: Synthetic polypeptide
AAEQNPIYWARYADWLFTTPLLLLALALLVDADEGT

SEQ ID NO: 16 - protein, 36 aa, synthetic construct
  REGION 1..36: note = Description of Artificial Sequence: Synthetic polypeptide
AAEQNPIYWARYAAWLFTTPLLLLDLALLVDADEGT

SEQ ID NO: 17 - protein, 36 aa, synthetic construct
  REGION 1..36: note = Description of Artificial Sequence: Synthetic polypeptide
AAEQNPIYWARYADWLFTTALLLLDLALLVDADEGT

SEQ ID NO: 18 - protein, 36 aa, synthetic construct
  REGION 1..36: note = Description of Artificial Sequence: Synthetic polypeptide
AAEQNPIYWARYADWLFTTPLLLLELALLVDADEGT

SEQ ID NO: 19 - protein, 36 aa, synthetic construct
  REGION 1..36: note = Description of Artificial Sequence: Synthetic polypeptide
AAEQNPIYWARYAEWLFTTPLLLLDLALLVDADEGT

SEQ ID NO: 20 - protein, 39 aa, synthetic construct
  REGION 1..39: note = Description of Artificial Sequence: Synthetic polypeptide
AAEQNPIIYWARYADWLFTDLPLLLLDLLALLVDADEGT

SEQ ID NO: 21 - protein, 37 aa, synthetic construct
  REGION 1..37: note = Description of Artificial Sequence: Synthetic polypeptide
GEQNPIYWAQYADWLFTTPLLLLDLALLVDADEGTCG

SEQ ID NO: 22 - protein, 38 aa, synthetic construct
  REGION 1..38: note = Description of Artificial Sequence: Synthetic polypeptide
GGEQNPIYWARYADWLFTTPLLLDLLALLVDADEGTCG

SEQ ID NO: 23 - protein, 38 aa, synthetic construct
  REGION 1..38: note = Description of Artificial Sequence: Synthetic polypeptide
GGEQNPIYWARYADWLFTTPLLLLLDALLVDADEGTCG

SEQ ID NO: 24 - protein, 38 aa, synthetic construct
  REGION 1..38: note = Description of Artificial Sequence: Synthetic polypeptide
GGEQNPIYWARYDAWLFTTPLLLLDLALLVDADEGTCG

SEQ ID NO: 25 - protein, 38 aa, synthetic construct
  REGION 1..38: note = Description of Artificial Sequence: Synthetic polypeptide
GGEQNPIYWARYAWDLFTTPLLLLDLALLVDADEGTCG

SEQ ID NO: 26 - protein, 36 aa, synthetic construct
  REGION 1..36: note = Description of Artificial Sequence: Synthetic polypeptide
AAEQNPIYWARYADWLFTTGLLLLDLALLVDADEGT

SEQ ID NO: 27 - protein, 37 aa, synthetic construct
  REGION 1..37: note = Description of Artificial Sequence: Synthetic polypeptide
DDDEDNPIYWARYADWLFTTPLLLLHGALLVDADECT

SEQ ID NO: 28 - protein, 38 aa, synthetic construct
  REGION 1..38: note = Description of Artificial Sequence: Synthetic polypeptide
DDDEDNPIYWARYAHWLFTTPLLLLHGALLVDADEGCT

SEQ ID NO: 29 - protein, 37 aa, synthetic construct
  REGION 1..37: note = Description of Artificial Sequence: Synthetic polypeptide
DDDEDNPIYWARYAHWLFTTPLLLLHGALLVNADECT

SEQ ID NO: 30 - protein, 37 aa, synthetic construct
  REGION 1..37: note = Description of Artificial Sequence: Synthetic polypeptide
DDDEDNPIYWARYAHWLFTTPLLLLHGALLVNANECT

SEQ ID NO: 31 - protein, 34 aa, synthetic construct
  REGION 1..34: note = Description of Artificial Sequence: Synthetic polypeptide
AEQNPIYWARYADFLFTTPLLLLDLALLVDADET

SEQ ID NO: 32 - protein, 35 aa, synthetic construct
  REGION 1..35: note = Description of Artificial Sequence: Synthetic polypeptide
AEQNPIYFARYADWLFTTPLLLLDLALLVDADEGT

SEQ ID NO: 33 - protein, 34 aa, synthetic construct
  REGION 1..34: note = Description of Artificial Sequence: Synthetic polypeptide
AEQNPIYFARYADFLFTTPLLLLDLALLWDADET

SEQ ID NO: 34 - protein, 32 aa, synthetic construct
  REGION 1..32: note = Description of Artificial Sequence: Synthetic polypeptide
AKEDQNPYWARYADWLFTTPLLLLDLALLVDG

SEQ ID NO: 35 - protein, 32 aa, synthetic construct
  REGION 1..32: note = Description of Artificial Sequence: Synthetic polypeptide
ACEDQNPYWARYADWLFTTPLLLLDLALLVDG

SEQ ID NO: 36 - protein, 32 aa, synthetic construct
  REGION 1..32: note = Description of Artificial Sequence: Synthetic polypeptide
AEDQNPYWARYADWLFTTPLLLLDLALLVDCG

SEQ ID NO: 37 - protein, 32 aa, synthetic construct
  REGION 1..32: note = Description of Artificial Sequence: Synthetic polypeptide
AEDQNPYWARYADWLFTTPLLLLELALLVECG

SEQ ID NO: 38 - protein, 30 aa, synthetic construct
  REGION 1..30: note = Description of Artificial Sequence: Synthetic polypeptide
AKEDQNPYWRAYADLFTPLTLLDLLALWDG

SEQ ID NO: 39 - protein, 30 aa, synthetic construct
  REGION 1..30: note = Description of Artificial Sequence: Synthetic polypeptide
ACEDQNPYWRAYADLFTPLTLLDLLALWDG

SEQ ID NO: 40 - protein, 27 aa, synthetic construct
  REGION 1..27: note = Description of Artificial Sequence: Synthetic peptide
ACDDQNPWRAYLDLLFPTDTLLLDLLW

SEQ ID NO: 41 - protein, 34 aa, synthetic construct
  REGION 1..34: note = Description of Artificial Sequence: Synthetic polypeptide
TEDADVLLALDLLLLPTTFLWDAYRAWYPNQECA

SEQ ID NO: 42 - protein, 20 aa, synthetic construct
  REGION 1..20: note = Description of Artificial Sequence: Synthetic peptide
AEQNPIYWARYADWLFTTPL

SEQ ID NO: 43 - protein, 21 aa, synthetic construct
  REGION 1..21: note = Description of Artificial Sequence: Synthetic peptide
AEQNPIYWARYADWLFTTPCL

SEQ ID NO: 44 - protein, 21 aa, synthetic construct
  REGION 1..21: note = Description of Artificial Sequence: Synthetic peptide
ACEQNPIYWARYADWLFTTPL

SEQ ID NO: 45 - protein, 20 aa, synthetic construct
  REGION 1..20: note = Description of Artificial Sequence: Synthetic peptide
AEQNPIYFARYADWLFTTPL

SEQ ID NO: 46 - protein, 21 aa, synthetic construct
  REGION 1..21: note = Description of Artificial Sequence: Synthetic peptide
KEDQNPWARYADLLFPTTLAW

SEQ ID NO: 47 - protein, 22 aa, synthetic construct
  REGION 1..22: note = Description of Artificial Sequence: Synthetic peptide
ACEDQNPWARYADLLFPTTLAW

SEQ ID NO: 48 - protein, 24 aa, synthetic construct
  REGION 1..24: note = Description of Artificial Sequence: Synthetic peptide
ACEDQNPWARYADWLFPTTLLLLD

SEQ ID NO: 49 - protein, 22 aa, synthetic construct
  REGION 1..22: note = Description of Artificial Sequence: Synthetic peptide
ACEEQNPWARYAELLFPTTLAW

SEQ ID NO: 50 - protein, 24 aa, synthetic construct
  REGION 1..24: note = Description of Artificial Sequence: Synthetic peptide
ACEEQNPWARYAEWLFPTTLLLLE

SEQ ID NO: 51 - protein, 25 aa, synthetic construct
  REGION 1..25: note = Description of Artificial Sequence: Synthetic peptide
ACEEQNPWARYLEWLFPTETLLLEL

SEQ ID NO: 52 - protein, 36 aa, synthetic construct; identical to SEQ ID NO: 3
  REGION 1..36: note = Description of Artificial Sequence: Synthetic polypeptide

SEQ ID NO: 53 - protein, 35 aa, synthetic construct
  REGION 1..35: note = Description of Artificial Sequence: Synthetic polypeptide
ACEQNPIYWARYADWLFTTPLLLLDLALLVDADET

SEQ ID NO: 54 - protein, 38 aa, synthetic construct; identical to SEQ ID NO: 5
  REGION 1..38: note = Description of Artificial Sequence: Synthetic polypeptide

SEQ ID NO: 55 - protein, 36 aa, synthetic construct
  REGION 1..36: note = Description of Artificial Sequence: Synthetic polypeptide
AEQNPIYWARYADWLFTTPLLLLDLALLVDADEGCT

SEQ ID NO: 56 - protein, 38 aa, synthetic construct; identical to SEQ ID NO: 6
  REGION 1..38: note = Description of Artificial Sequence: Synthetic polypeptide

SEQ ID NO: 57 - protein, 36 aa, synthetic construct; identical to SEQ ID NO: 8
  REGION 1..36: note = Description of Artificial Sequence: Synthetic polypeptide

SEQ ID NO: 58 - protein, 36 aa, synthetic construct; identical to SEQ ID NO: 9
  REGION 1..36: note = Description of Artificial Sequence: Synthetic polypeptide

SEQ ID NO: 59 - protein, 36 aa, synthetic construct; identical to SEQ ID NO: 11
  REGION 1..36: note = Description of Artificial Sequence: Synthetic polypeptide

SEQ ID NO: 60 - protein, 36 aa, synthetic construct; identical to SEQ ID NO: 17
  REGION 1..36: note = Description of Artificial Sequence: Synthetic polypeptide

SEQ ID NO: 61 - protein, 37 aa, synthetic construct
  REGION 1..37: note = Description of Artificial Sequence: Synthetic polypeptide
ACAEQNPIYWARYADWLFTTGLLLLDLALLVDADEGT

SEQ ID NO: 62 - protein, 34 aa, synthetic construct; identical to SEQ ID NO: 31
  REGION 1..34: note = Description of Artificial Sequence: Synthetic polypeptide

SEQ ID NO: 63 - protein, 35 aa, synthetic construct; identical to SEQ ID NO: 32
  REGION 1..35: note = Description of Artificial Sequence: Synthetic polypeptide

SEQ ID NO: 64 - protein, 34 aa, synthetic construct; identical to SEQ ID NO: 33
  REGION 1..34: note = Description of Artificial Sequence: Synthetic polypeptide

SEQ ID NO: 65 - protein, 32 aa, synthetic construct; identical to SEQ ID NO: 34
  REGION 1..32: note = Description of Artificial Sequence: Synthetic polypeptide

SEQ ID NO: 66 - protein, 32 aa, synthetic construct; identical to SEQ ID NO: 35
  REGION 1..32: note = Description of Artificial Sequence: Synthetic polypeptide

SEQ ID NO: 67 - protein, 31 aa, synthetic construct
  REGION 1..31: note = Description of Artificial Sequence: Synthetic polypeptide
AEDQNPYWARYADWLFTTPLLLLDLALLVDG

SEQ ID NO: 68 - protein, 32 aa, synthetic construct; identical to SEQ ID NO: 37
  REGION 1..32: note = Description of Artificial Sequence: Synthetic polypeptide

SEQ ID NO: 69 - protein, 30 aa, synthetic construct; identical to SEQ ID NO: 38
  REGION 1..30: note = Description of Artificial Sequence: Synthetic polypeptide

SEQ ID NO: 70 - protein, 30 aa, synthetic construct; identical to SEQ ID NO: 39
  REGION 1..30: note = Description of Artificial Sequence: Synthetic polypeptide

SEQ ID NO: 71 - protein, 32 aa, synthetic construct
  REGION 1..32: note = Description of Artificial Sequence: Synthetic polypeptide
AKEDQNDPYWARYADWLFTTPLLLLDLALLVG

SEQ ID NO: 72 - protein, 34 aa, synthetic construct; identical to SEQ ID NO: 41
  REGION 1..34: note = Description of Artificial Sequence: Synthetic polypeptide

SEQ ID NO: 73 - protein, 36 aa, unidentified; identical to SEQ ID NO: 3
  REGION 1..36: note = Description of Unknown: Wild-type pH-sensitive membrane polypeptide

SEQ ID NO: 74 - protein, 20 aa, synthetic construct
  REGION 1..20: note = Description of Artificial Sequence: Synthetic peptide
AEQNPIYWARYADWLFTTPL

SEQ ID NO: 75 - protein, 21 aa, synthetic construct
  REGION 1..21: note = Description of Artificial Sequence: Synthetic peptide
AEQNPIYWARYADWLFTTPCL

SEQ ID NO: 76 - protein, 21 aa, synthetic construct
  REGION 1..21: note = Description of Artificial Sequence: Synthetic peptide
ACEQNPIYWARYADWLFTTPL

SEQ ID NO: 77 - protein, 21 aa, synthetic construct
  REGION 1..21: note = Description of Artificial Sequence: Synthetic peptide
ACEQNPIYFARYADWLFTTPL

SEQ ID NO: 78 - protein, 27 aa, synthetic construct
  REGION 1..27: note = Description of Artificial Sequence: Synthetic peptide
ACDDQNPWRAYLDLLFPTDTLLLDLLW

SEQ ID NO: 79 - protein, 27 aa, synthetic construct
  REGION 1..27: note = Description of Artificial Sequence: Synthetic peptide
ACEEQNPWRAYLELLFPTETLLLELLW

SEQ ID NO: 80 - protein, 25 aa, synthetic construct
  REGION 1..25: note = Description of Artificial Sequence: Synthetic peptide
ACDDQNPWARYLDWLFPTDTLLLDL

SEQ ID NO: 81 - protein, 24 aa, synthetic construct
  REGION 1..24: note = Description of Artificial Sequence: Synthetic peptide
CDNNNPWRAYLDLLFPTDTLLLDW

SEQ ID NO: 82 - protein, 25 aa, synthetic construct
  REGION 1..25: note = Description of Artificial Sequence: Synthetic peptide
ACEEQNPWARYLEWLFPTETLLLEL

SEQ ID NO: 83 - protein, 24 aa, synthetic construct
  REGION 1..24: note = Description of Artificial Sequence: Synthetic peptide
ACEDQNPWARYADWLFPTTLLLLD

SEQ ID NO: 84 - protein, 24 aa, synthetic construct
  REGION 1..24: note = Description of Artificial Sequence: Synthetic peptide
ACEEQNPWARYAEWLFPTTLLLLE

SEQ ID NO: 85 - protein, 22 aa, synthetic construct
  REGION 1..22: note = Description of Artificial Sequence: Synthetic peptide
ACEDQNPWARYADLLFPTTLAW

SEQ ID NO: 86 - protein, 21 aa, synthetic construct
  REGION 1..21: note = Description of Artificial Sequence: Synthetic peptide
ACEDQNPWARYAELLFPTTLW

SEQ ID NO: 87 - protein, 20 aa, synthetic construct
  REGION 1..20: note = Description of Artificial Sequence: Synthetic peptide
KEDQNPWARYADLLFPTTLW

SEQ ID NO: 88 - protein, 37 aa, synthetic construct
  REGION 1..37: note = Description of Artificial Sequence: Synthetic polypeptide
DDDEDNPIYWARYAHWLFTTPLLLLHGALLVDADECT

SEQ ID NO: 89 - protein, 37 aa, synthetic construct
  REGION 1..37: note = Description of Artificial Sequence: Synthetic polypeptide
DDDEDNPIYWARYAHWLFTTPLLLLDGALLVDADECT

SEQ ID NO: 90 - protein, 37 aa, synthetic construct; identical to SEQ ID NO: 29
  REGION 1..37: note = Description of Artificial Sequence: Synthetic polypeptide

SEQ ID NO: 91 - protein, 37 aa, synthetic construct; identical to SEQ ID NO: 30
  REGION 1..37: note = Description of Artificial Sequence: Synthetic polypeptide

SEQ ID NO: 92 - protein, 37 aa, synthetic construct; identical to SEQ ID NO: 27
  REGION 1..37: note = Description of Artificial Sequence: Synthetic polypeptide

SEQ ID NO: 93 - protein, 37 aa, synthetic construct; identical to SEQ ID NO: 7
  REGION 1..37: note = Description of Artificial Sequence: Synthetic polypeptide

SEQ ID NO: 94 - protein, 35 aa, synthetic construct; identical to SEQ ID NO: 53
  REGION 1..35: note = Description of Artificial Sequence: Synthetic polypeptide

SEQ ID NO: 95 - protein, 36 aa, synthetic construct; identical to SEQ ID NO: 8
  REGION 1..36: note = Description of Artificial Sequence: Synthetic polypeptide

SEQ ID NO: 96 - protein, 38 aa, synthetic construct; identical to SEQ ID NO: 22
  REGION 1..38: note = Description of Artificial Sequence: Synthetic polypeptide

SEQ ID NO: 97 - protein, 38 aa, synthetic construct; identical to SEQ ID NO: 23
  REGION 1..38: note = Description of Artificial Sequence: Synthetic polypeptide

SEQ ID NO: 98 - protein, 38 aa, synthetic construct; identical to SEQ ID NO: 25
  REGION 1..38: note = Description of Artificial Sequence: Synthetic polypeptide

SEQ ID NO: 99 - protein, 38 aa, synthetic construct
  REGION 1..38: note = Description of Artificial Sequence: Synthetic polypeptide
AAEQNPIYWARYAEWLFTTPLLLLDLALLVDADEGTCG

SEQ ID NO: 100 - protein, 38 aa, synthetic construct
  REGION 1..38: note = Description of Artificial Sequence: Synthetic polypeptide
AAEQNPIYWARYAEWLFTTPLLLLELALLVDADEGTCG

SEQ ID NO: 101 - protein, 38 aa, synthetic construct; identical to SEQ ID NO: 24
  REGION 1..38: note = Description of Artificial Sequence: Synthetic polypeptide

SEQ ID NO: 102 - protein, 38 aa, synthetic construct
  REGION 1..38: note = Description of Artificial Sequence: Synthetic polypeptide
GGEQNPIYWAQYDAWLFTTPLLLLDLALLVDADEGTCG

SEQ ID NO: 103 - protein, 38 aa, synthetic construct
  REGION 1..38: note = Description of Artificial Sequence: Synthetic polypeptide
GGEQNPIYWAQDYAWLFTTPLLLLDLALLVDADEGTCG

SEQ ID NO: 104 - protein, 38 aa, synthetic construct
  REGION 1..38: note = Description of Artificial Sequence: Synthetic polypeptide
AAEQNPIYWARYAAWLFTTPLLLLDLALLVDADEGTCG

SEQ ID NO: 105 - protein, 37 aa, synthetic construct; identical to SEQ ID NO: 12
  REGION 1..37: note = Description of Artificial Sequence: Synthetic polypeptide

SEQ ID NO: 106 - protein, 37 aa, synthetic construct; identical to SEQ ID NO: 30
  REGION 1..37: note = Description of Artificial Sequence: Synthetic polypeptide

SEQ ID NO: 107 - protein, 37 aa, synthetic construct; identical to SEQ ID NO: 29
  REGION 1..37: note = Description of Artificial Sequence: Synthetic polypeptide

SEQ ID NO: 108 - protein, 37 aa, synthetic construct; identical to SEQ ID NO: 27
  REGION 1..37: note = Description of Artificial Sequence: Synthetic polypeptide

SEQ ID NO: 109 - protein, 37 aa, synthetic construct; identical to SEQ ID NO: 88
  REGION 1..37: note = Description of Artificial Sequence: Synthetic polypeptide

SEQ ID NO: 110 - protein, 37 aa, synthetic construct; identical to SEQ ID NO: 89
  REGION 1..37: note = Description of Artificial Sequence: Synthetic polypeptide

SEQ ID NO: 111 - protein, 36 aa, synthetic construct; identical to SEQ ID NO: 14
  REGION 1..36: note = Description of Artificial Sequence: Synthetic polypeptide

SEQ ID NO: 112 - protein, 38 aa, synthetic construct
  REGION 1..38: note = Description of Artificial Sequence: Synthetic polypeptide
AAEQNPIYWARYADWLFTTPLLLLELALLVDADEGTCG

SEQ ID NO: 113 - protein, 38 aa, synthetic construct; identical to SEQ ID NO: 100
  REGION 1..38: note = Description of Artificial Sequence: Synthetic polypeptide

SEQ ID NO: 114 - protein, 39 aa, synthetic construct
  REGION 1..39: note = Description of Artificial Sequence: Synthetic polypeptide
AAEQNPIYWARYADWLFTTPLLLLELALLVDADEGTKCG

SEQ ID NO: 115 - protein, 38 aa, synthetic construct
  REGION 1..38: note = Description of Artificial Sequence: Synthetic polypeptide
GGEQNPIYWAQYADWLFTTPLLLLDLALLVDADEGTCG

SEQ ID NO: 116 - protein, 38 aa, synthetic construct; identical to SEQ ID NO: 102
  REGION 1..38: note = Description of Artificial Sequence: Synthetic polypeptide

SEQ ID NO: 117 - protein, 38 aa, synthetic construct; identical to SEQ ID NO: 103
  REGION 1..38: note = Description of Artificial Sequence: Synthetic polypeptide

SEQ ID NO: 118 - protein, 36 aa, synthetic construct; identical to SEQ ID NO: 14
  REGION 1..36: note = Description of Artificial Sequence: Synthetic polypeptide

SEQ ID NO: 119 - protein, 37 aa, synthetic construct; identical to SEQ ID NO: 29
  REGION 1..37: note = Description of Artificial Sequence: Synthetic polypeptide

SEQ ID NO: 120 - protein, 37 aa, synthetic construct; identical to SEQ ID NO: 30
  REGION 1..37: note = Description of Artificial Sequence: Synthetic polypeptide

SEQ ID NO: 121 - protein, 37 aa, synthetic construct; identical to SEQ ID NO: 13
  REGION 1..37: note = Description of Artificial Sequence: Synthetic polypeptide

SEQ ID NO: 122 - protein, 38 aa, synthetic construct; identical to SEQ ID NO: 103
  REGION 1..38: note = Description of Artificial Sequence: Synthetic polypeptide

SEQ ID NO: 123 - protein, 38 aa, synthetic construct; identical to SEQ ID NO: 102
  REGION 1..38: note = Description of Artificial Sequence: Synthetic polypeptide

SEQ ID NO: 124 - protein, 38 aa, synthetic construct; identical to SEQ ID NO: 115
  REGION 1..38: note = Description of Artificial Sequence: Synthetic polypeptide

SEQ ID NO: 125 - protein, 38 aa, synthetic construct; identical to SEQ ID NO: 104
  REGION 1..38: note = Description of Artificial Sequence: Synthetic polypeptide

SEQ ID NO: 126 - protein, 38 aa, synthetic construct
  REGION 1..38: note = Description of Artificial Sequence: Synthetic polypeptide
AAEQNPIYWARYADWLFTDLPLLLLDLLALLVDADEGT

SEQ ID NO: 127 - protein, 38 aa, synthetic construct; identical to SEQ ID NO: 23
  REGION 1..38: note = Description of Artificial Sequence: Synthetic polypeptide

SEQ ID NO: 128 - protein, 38 aa, synthetic construct; identical to SEQ ID NO: 22
  REGION 1..38: note = Description of Artificial Sequence: Synthetic polypeptide

SEQ ID NO: 129 - protein, 36 aa, synthetic construct; identical to SEQ ID NO: 26
  REGION 1..36: note = Description of Artificial Sequence: Synthetic polypeptide

SEQ ID NO: 130 - protein, 38 aa, synthetic construct; identical to SEQ ID NO: 104
  REGION 1..38: note = Description of Artificial Sequence: Synthetic polypeptide

SEQ ID NO: 131 - protein, 38 aa, synthetic construct; identical to SEQ ID NO: 102
  REGION 1..38: note = Description of Artificial Sequence: Synthetic polypeptide

SEQ ID NO: 132 - protein, 38 aa, synthetic construct; identical to SEQ ID NO: 103
  REGION 1..38: note = Description of Artificial Sequence: Synthetic polypeptide

SEQ ID NO: 133 - protein, 38 aa, synthetic construct; identical to SEQ ID NO: 24
  REGION 1..38: note = Description of Artificial Sequence: Synthetic polypeptide

SEQ ID NO: 134 - protein, 38 aa, synthetic construct
  REGION 1..38: note = Description of Artificial Sequence: Synthetic polypeptide
AAEQNPIYWARYADWLFTTPLLLLALALLVDADEGTCG

SEQ ID NO: 135 - protein, 39 aa, synthetic construct; identical to SEQ ID NO: 10
  REGION 1..39: note = Description of Artificial Sequence: Synthetic polypeptide
  MOD_RES 37: note = Lys(rhodamine)
  MOD_RES 38: note = Cys(phalloidin)

SEQ ID NO: 136 - protein, 39 aa, synthetic construct; identical to SEQ ID NO: 114
  REGION 1..39: note = Description of Artificial Sequence: Synthetic polypeptide
  MOD_RES 37: note = Lys(rhodamine)
  MOD_RES 38: note = Cys(phalloidin)

SEQ ID NO: 137 - protein, 38 aa, synthetic construct; identical to SEQ ID NO: 5
  REGION 1..38: note = Description of Artificial Sequence: Synthetic polypeptide
  MOD_RES 37: note = Cys(phalloidin)

SEQ ID NO: 138 - protein, 38 aa, synthetic construct; identical to SEQ ID NO: 5
  REGION 1..38: note = Description of Artificial Sequence: Synthetic polypeptide
  MOD_RES 37: note = Cys(phalloidin)

SEQ ID NO: 139 - protein, 38 aa, synthetic construct; identical to SEQ ID NO: 6
  REGION 1..38: note = Description of Artificial Sequence: Synthetic polypeptide

SEQ ID NO: 140 - protein, 35 aa, synthetic construct; identical to SEQ ID NO: 53
  REGION 1..35: note = Description of Artificial Sequence: Synthetic polypeptide

SEQ ID NO: 141 - protein, 37 aa, synthetic construct; identical to SEQ ID NO: 7
  REGION 1..37: note = Description of Artificial Sequence: Synthetic polypeptide

SEQ ID NO: 142 - protein, 36 aa, synthetic construct; identical to SEQ ID NO: 8
  REGION 1..36: note = Description of Artificial Sequence: Synthetic polypeptide

SEQ ID NO: 143 - protein, 36 aa, synthetic construct; identical to SEQ ID NO: 14
  REGION 1..36: note = Description of Artificial Sequence: Synthetic polypeptide

SEQ ID NO: 144 - protein, 37 aa, synthetic construct; identical to SEQ ID NO: 29
  REGION 1..37: note = Description of Artificial Sequence: Synthetic polypeptide

SEQ ID NO: 145 - protein, 37 aa, synthetic construct; identical to SEQ ID NO: 30
  REGION 1..37: note = Description of Artificial Sequence: Synthetic polypeptide

SEQ ID NO: 146 - protein, 38 aa, synthetic construct; identical to SEQ ID NO: 6
  REGION 1..38: note = Description of Artificial Sequence: Synthetic polypeptide

SEQ ID NO: 147 - protein, 38 aa, synthetic construct; identical to SEQ ID NO: 5
  REGION 1..38: note = Description of Artificial Sequence: Synthetic polypeptide
  MOD_RES 37: note = Cys(phalloidin)

SEQ ID NO: 148 - protein, 39 aa, synthetic construct; identical to SEQ ID NO: 114
  REGION 1..39: note = Description of Artificial Sequence: Synthetic polypeptide
  MOD_RES 37: note = Lys(rhodamine)
  MOD_RES 38: note = Cys(phalloidin)

SEQ ID NO: 149 - protein, 39 aa, synthetic construct; identical to SEQ ID NO: 10
  REGION 1..39: note = Description of Artificial Sequence: Synthetic polypeptide
  MOD_RES 37: note = Lys(rhodamine)
  MOD_RES 38: note = Cys(phalloidin)

SEQ ID NO: 150 - protein, 37 aa, synthetic construct; identical to SEQ ID NO: 88
  REGION 1..37: note = Description of Artificial Sequence: Synthetic polypeptide

SEQ ID NO: 151 - protein, 37 aa, synthetic construct; identical to SEQ ID NO: 89
  REGION 1..37: note = Description of Artificial Sequence: Synthetic polypeptide

SEQ ID NO: 152 - protein, 37 aa, synthetic construct; identical to SEQ ID NO: 29
  REGION 1..37: note = Description of Artificial Sequence: Synthetic polypeptide

SEQ ID NO: 153 - protein, 37 aa, synthetic construct; identical to SEQ ID NO: 30
  REGION 1..37: note = Description of Artificial Sequence: Synthetic polypeptide

SEQ ID NO: 154 - protein, 37 aa, synthetic construct; identical to SEQ ID NO: 27
  REGION 1..37: note = Description of Artificial Sequence: Synthetic polypeptide

SEQ ID NO: 155 - protein, 37 aa, synthetic construct; identical to SEQ ID NO: 27
  REGION 1..37: note = Description of Artificial Sequence: Synthetic polypeptide

SEQ ID NO: 156 - protein, 37 aa, synthetic construct; identical to SEQ ID NO: 89
  REGION 1..37: note = Description of Artificial Sequence: Synthetic polypeptide

SEQ ID NO: 157 - protein, 37 aa, synthetic construct; identical to SEQ ID NO: 88
  REGION 1..37: note = Description of Artificial Sequence: Synthetic polypeptide

SEQ ID NO: 158 - protein, 37 aa, synthetic construct; identical to SEQ ID NO: 29
  REGION 1..37: note = Description of Artificial Sequence: Synthetic polypeptide

SEQ ID NO: 159 - protein, 37 aa, synthetic construct; identical to SEQ ID NO: 30
  REGION 1..37: note = Description of Artificial Sequence: Synthetic polypeptide

SEQ ID NO: 160 - protein, 37 aa, synthetic construct; identical to SEQ ID NO: 30
  REGION 1..37: note = Description of Artificial Sequence: Synthetic polypeptide

SEQ ID NO: 161 - protein, 37 aa, synthetic construct; identical to SEQ ID NO: 29
  REGION 1..37: note = Description of Artificial Sequence: Synthetic polypeptide

SEQ ID NO: 162 - protein, 37 aa, synthetic construct; identical to SEQ ID NO: 27
  REGION 1..37: note = Description of Artificial Sequence: Synthetic polypeptide

SEQ ID NO: 163 - protein, 37 aa, synthetic construct; identical to SEQ ID NO: 88
  REGION 1..37: note = Description of Artificial Sequence: Synthetic polypeptide

SEQ ID NO: 164 - protein, 37 aa, synthetic construct; identical to SEQ ID NO: 89
  REGION 1..37: note = Description of Artificial Sequence: Synthetic polypeptide

SEQ ID NO: 165 - protein, 36 aa, synthetic construct; identical to SEQ ID NO: 14
  REGION 1..36: note = Description of Artificial Sequence: Synthetic polypeptide

SEQ ID NO: 166 - protein, 37 aa, synthetic construct; identical to SEQ ID NO: 29
  REGION 1..37: note = Description of Artificial Sequence: Synthetic polypeptide

SEQ ID NO: 167 - protein, 37 aa, synthetic construct; identical to SEQ ID NO: 27
  REGION 1..37: note = Description of Artificial Sequence: Synthetic polypeptide

SEQ ID NO: 168 - protein, 37 aa, synthetic construct; identical to SEQ ID NO: 88
  REGION 1..37: note = Description of Artificial Sequence: Synthetic polypeptide

SEQ ID NO: 169 - protein, 37 aa, synthetic construct; identical to SEQ ID NO: 89
  REGION 1..37: note = Description of Artificial Sequence: Synthetic polypeptide

SEQ ID NO: 170 - protein, 37 aa, synthetic construct; identical to SEQ ID NO: 30
  REGION 1..37: note = Description of Artificial Sequence: Synthetic polypeptide

SEQ ID NO: 171 - protein, 37 aa, synthetic construct; identical to SEQ ID NO: 89
  REGION 1..37: note = Description of Artificial Sequence: Synthetic polypeptide

SEQ ID NO: 172 - protein, 37 aa, synthetic construct; identical to SEQ ID NO: 27
  REGION 1..37: note = Description of Artificial Sequence: Synthetic polypeptide

SEQ ID NO: 173 - protein, 37 aa, synthetic construct; identical to SEQ ID NO: 88
  REGION 1..37: note = Description of Artificial Sequence: Synthetic polypeptide

SEQ ID NO: 174 - protein, 37 aa, synthetic construct; identical to SEQ ID NO: 29
  REGION 1..37: note = Description of Artificial Sequence: Synthetic polypeptide

SEQ ID NO: 175 - protein, 37 aa, synthetic construct; identical to SEQ ID NO: 30
  REGION 1..37: note = Description of Artificial Sequence: Synthetic polypeptide

SEQ ID NO: 176 - protein, 36 aa, synthetic construct; identical to SEQ ID NO: 26
  REGION 1..36: note = Description of Artificial Sequence: Synthetic polypeptide

SEQ ID NO: 177 - protein, 38 aa, synthetic construct; identical to SEQ ID NO: 25
  REGION 1..38: note = Description of Artificial Sequence: Synthetic polypeptide

SEQ ID NO: 178 - protein, 38 aa, synthetic construct; identical to SEQ ID NO: 24
  REGION 1..38: note = Description of Artificial Sequence: Synthetic polypeptide

SEQ ID NO: 179 - protein, 38 aa, synthetic construct; identical to SEQ ID NO: 102
  REGION 1..38: note = Description of Artificial Sequence: Synthetic polypeptide

SEQ ID NO: 180 - protein, 38 aa, synthetic construct; identical to SEQ ID NO: 103
  REGION 1..38: note = Description of Artificial Sequence: Synthetic polypeptide

SEQ ID NO: 181 - protein, 38 aa, synthetic construct; identical to SEQ ID NO: 104
  REGION 1..38: note = Description of Artificial Sequence: Synthetic polypeptide

SEQ ID NO: 182 - protein, 38 aa, synthetic construct; identical to SEQ ID NO: 23
  REGION 1..38: note = Description of Artificial Sequence: Synthetic polypeptide

SEQ ID NO: 183 - protein, 38 aa, synthetic construct; identical to SEQ ID NO: 22
  REGION 1..38: note = Description of Artificial Sequence: Synthetic polypeptide

SEQ ID NO: 184 - protein, 38 aa, synthetic construct; identical to SEQ ID NO: 22
  REGION 1..38: note = Description of Artificial Sequence: Synthetic polypeptide

SEQ ID NO: 185 - protein, 38 aa, synthetic construct; identical to SEQ ID NO: 23
  REGION 1..38: note = Description of Artificial Sequence: Synthetic polypeptide

SEQ ID NO: 186 - protein, 38 aa, synthetic construct; identical to SEQ ID NO: 115
  REGION 1..38: note = Description of Artificial Sequence: Synthetic polypeptide

SEQ ID NO: 187 - protein, 38 aa, synthetic construct; identical to SEQ ID NO: 102
  REGION 1..38: note = Description of Artificial Sequence: Synthetic polypeptide

SEQ ID NO: 188 - protein, 38 aa, synthetic construct; identical to SEQ ID NO: 103
  REGION 1..38: note = Description of Artificial Sequence: Synthetic polypeptide

SEQ ID NO: 189 - protein, 38 aa, synthetic construct; identical to SEQ ID NO: 102
  REGION 1..38: note = Description of Artificial Sequence: Synthetic polypeptide

SEQ ID NO: 190 - protein, 38 aa, synthetic construct; identical to SEQ ID NO: 103
  REGION 1..38: note = Description of Artificial Sequence: Synthetic polypeptide

SEQ ID NO: 191 - protein, 38 aa, synthetic construct; identical to SEQ ID NO: 115
  REGION 1..38: note = Description of Artificial Sequence: Synthetic polypeptide

SEQ ID NO: 192 - protein, 38 aa, synthetic construct; identical to SEQ ID NO: 104
  REGION 1..38: note = Description of Artificial Sequence: Synthetic polypeptide

SEQ ID NO: 193 - protein, 38 aa, synthetic construct; identical to SEQ ID NO: 103
  REGION 1..38: note = Description of Artificial Sequence: Synthetic polypeptide

SEQ ID NO: 194 - protein, 38 aa, synthetic construct; identical to SEQ ID NO: 102
  REGION 1..38: note = Description of Artificial Sequence: Synthetic polypeptide

SEQ ID NO: 195 - protein, 38 aa, synthetic construct; identical to SEQ ID NO: 115
  REGION 1..38: note = Description of Artificial Sequence: Synthetic polypeptide

SEQ ID NO: 196 - protein, 38 aa, synthetic construct; identical to SEQ ID NO: 104
  REGION 1..38: note = Description of Artificial Sequence: Synthetic polypeptide

SEQ ID NO: 197 - protein, 39 aa, synthetic construct; identical to SEQ ID NO: 114
  REGION 1..39: note = Description of Artificial Sequence: Synthetic polypeptide

SEQ ID NO: 198 - protein, 6 aa, synthetic construct
  REGION 1..6: note = Description of Artificial Sequence: Synthetic peptide
  MOD_RES 4: note = Lys(rhodamine)
  MOD_RES 5: note = Cys(phalloidin)
EGTKCG

SEQ ID NO: 199 - protein, 39 aa, synthetic construct; identical to SEQ ID NO: 10
  REGION 1..39: note = Description of Artificial Sequence: Synthetic polypeptide
  MOD_RES 37: note = Lys(rhodamine)
  MOD_RES 38: note = Cys(phalloidin)

SEQ ID NO: 200 - protein, 37 aa, synthetic construct; identical to SEQ ID NO: 7
  REGION 1..37: note = Description of Artificial Sequence: Synthetic polypeptide

SEQ ID NO: 201 - protein, 38 aa, synthetic construct; identical to SEQ ID NO: 5
  REGION 1..38: note = Description of Artificial Sequence: Synthetic polypeptide
  MOD_RES 37: note = Cys(phalloidin)

SEQ ID NO: 202 - protein, 39 aa, synthetic construct; identical to SEQ ID NO: 10
  REGION 1..39: note = Description of Artificial Sequence: Synthetic polypeptide
  MOD_RES 37: note = Lys(rhodamine)
  MOD_RES 38: note = Cys(phalloidin)

SEQ ID NO: 203 - protein, 39 aa, synthetic construct; identical to SEQ ID NO: 114
  REGION 1..39: note = Description of Artificial Sequence: Synthetic polypeptide
  MOD_RES 37: note = Lys(rhodamine)
  MOD_RES 38: note = Cys(phalloidin)

SEQ ID NO: 204 - protein, 38 aa, synthetic construct; identical to SEQ ID NO: 126
  REGION 1..38: note = Description of Artificial Sequence: Synthetic polypeptide

SEQ ID NO: 205 - protein, 38 aa, synthetic construct; identical to SEQ ID NO: 104
  REGION 1..38: note = Description of Artificial Sequence: Synthetic polypeptide

SEQ ID NO: 206 - protein, 38 aa, synthetic construct; identical to SEQ ID NO: 102
  REGION 1..38: note = Description of Artificial Sequence: Synthetic polypeptide

SEQ ID NO: 207 - protein, 38 aa, synthetic construct; identical to SEQ ID NO: 103
  REGION 1..38: note = Description of Artificial Sequence: Synthetic polypeptide

SEQ ID NO: 208 - protein, 38 aa, synthetic construct; identical to SEQ ID NO: 24
  REGION 1..38: note = Description of Artificial Sequence: Synthetic polypeptide

SEQ ID NO: 209 - protein, 38 aa, synthetic construct; identical to SEQ ID NO: 99
  REGION 1..38: note = Description of Artificial Sequence: Synthetic polypeptide

SEQ ID NO: 210 - protein, 38 aa, synthetic construct; identical to SEQ ID NO: 100
  REGION 1..38: note = Description of Artificial Sequence: Synthetic polypeptide

SEQ ID NO: 211 - protein, 38 aa, synthetic construct; identical to SEQ ID NO: 134
  REGION 1..38: note = Description of Artificial Sequence: Synthetic polypeptide

SEQ ID NO: 212 - protein, 38 aa, synthetic construct; identical to SEQ ID NO: 112
  REGION 1..38: note = Description of Artificial Sequence: Synthetic polypeptide

SEQ ID NO: 213 - protein, 38 aa, synthetic construct; identical to SEQ ID NO: 100
  REGION 1..38: note = Description of Artificial Sequence: Synthetic polypeptide

SEQ ID NO: 214 - protein, 39 aa, synthetic construct; identical to SEQ ID NO: 114
  REGION 1..39: note = Description of Artificial Sequence: Synthetic polypeptide
  MOD_RES 37: note = Lys(rhodamine)
  MOD_RES 38: note = Cys(phalloidin)

SEQ ID NO: 215 - protein, 37 aa, synthetic construct; identical to SEQ ID NO: 13
  REGION 1..37: note = Description of Artificial Sequence: Synthetic polypeptide

SEQ ID NO: 216 - protein, 37 aa, synthetic construct; identical to SEQ ID NO: 12
  REGION 1..37: note = Description of Artificial Sequence: Synthetic polypeptide

SEQ ID NO: 217 - protein, 36 aa, synthetic construct; identical to SEQ ID NO: 17
  REGION 1..36: note = Description of Artificial Sequence: Synthetic polypeptide

SEQ ID NO: 218 - protein, 22 aa, synthetic construct
  REGION 1..22: note = Description of Artificial Sequence: Synthetic peptide
AEQNPIYFARYADLLFPTTLAW

SEQ ID NO: 219 - protein, 22 aa, synthetic construct
  REGION 1..22: note = Description of Artificial Sequence: Synthetic peptide
AEQNPIYWARYADLLFPTTLAF

SEQ ID NO: 220 - protein, 22 aa, synthetic construct
  REGION 1..22: note = Description of Artificial Sequence: Synthetic peptide
AEQNPIYWARYADLLFPTTLAW

SEQ ID NO: 221 - protein, 35 aa, synthetic construct; identical to SEQ ID NO: 53
  REGION 1..35: note = Description of Artificial Sequence: Synthetic polypeptide

SEQ ID NO: 222 - skipped

SEQ ID NO: 223 - protein, 36 aa, synthetic construct; identical to SEQ ID NO: 3
  REGION 1..36: note = Description of Artificial Sequence: Synthetic polypeptide

SEQ ID NO: 224 - protein, 38 aa, synthetic construct; identical to SEQ ID NO: 5
  REGION 1..38: note = Description of Artificial Sequence: Synthetic polypeptide

SEQ ID NO: 225 - protein, 39 aa, synthetic construct; identical to SEQ ID NO: 10
  REGION 1..39: note = Description of Artificial Sequence: Synthetic polypeptide

SEQ ID NO: 226 - protein, 36 aa, synthetic construct; identical to SEQ ID NO: 11
  REGION 1..36: note = Description of Artificial Sequence: Synthetic polypeptide

SEQ ID NO: 227 - DNA, 18 bp, synthetic construct
  misc_feature 1..18: note = Description of Artificial Sequence: Synthetic oligonucleotide
  misc_feature 1..18: note = Peptide nucleic acid
  source 1..18: mol_type = other DNA
cctcttacctcagttaca

SEQ ID NO: 228 - DNA, 18 bp, synthetic construct
  misc_feature 1..18: note = Description of Artificial Sequence: Synthetic oligonucleotide
  misc_feature 1..18: note = Peptide nucleic acid
  source 1..18: mol_type = other DNA
cctcttacctcagttaca

SEQ ID NO: 229 - DNA, 18 bp, synthetic construct
  misc_feature 1..18: note = Description of Artificial Sequence: Synthetic oligonucleotide
  misc_feature 1..18: note = Peptide nucleic acid
  source 1..18: mol_type = other DNA
cctcttacctcagttaca

SEQ ID NO: 230 - DNA, 18 bp, synthetic construct
  misc_feature 1..18: note = Description of Artificial Sequence: Synthetic oligonucleotide
  misc_feature 1..18: note = Peptide nucleic acid
  source 1..18: mol_type = other DNA
cctcttacctcagttaca

SEQ ID NO: 231 - DNA, 18 bp, synthetic construct
  misc_feature 1..18: note = Description of Artificial Sequence: Synthetic oligonucleotide
  misc_feature 1..18: note = Peptide nucleic acid
  source 1..18: mol_type = other DNA
cctctgacctcatttaca

SEQ ID NO: 232 - DNA, 18 bp, synthetic construct
  misc_feature 1..18: note = Description of Artificial Sequence: Synthetic oligonucleotide
  misc_feature 1..18: note = Peptide nucleic acid
  source 1..18: mol_type = other DNA
cctcttacctcagttaca

SEQ ID NO: 233 - DNA, 18 bp, synthetic construct
  misc_feature 1..18: note = Description of Artificial Sequence: Synthetic oligonucleotide
  misc_feature 1..18: note = Peptide nucleic acid
  source 1..18: mol_type = other DNA
cctctgacctcatttaca

SEQ ID NO: 234 - DNA, 18 bp, synthetic construct
  misc_feature 1..18: note = Description of Artificial Sequence: Synthetic oligonucleotide
  misc_feature 1..18: note = Peptide nucleic acid
  source 1..18: mol_type = other DNA
cctcttacctcagttaca

SEQ ID NO: 235 - protein, 38 aa, unidentified; identical to SEQ ID NO: 5
  REGION 1..38: note = Description of Unknown: pH-sensitive membrane polypeptide

SEQ ID NO: 236 - protein, 31 aa, synthetic construct
  REGION 1..31: note = Description of Artificial Sequence: Synthetic polypeptide
AEDQNPYWARYDWLFTTPLLLLDLALLVDCG

SEQ ID NO: 237 - protein, 32 aa, synthetic construct; identical to SEQ ID NO: 37
  REGION 1..32: note = Description of Artificial Sequence: Synthetic polypeptide

SEQ ID NO: 238 - protein, 36 aa, synthetic construct; identical to SEQ ID NO: 55
  REGION 1..36: note = Description of Artificial Sequence: Synthetic polypeptide

SEQ ID NO: 239 - protein, 35 aa, synthetic construct; identical to SEQ ID NO: 53
  REGION 1..35: note = Description of Artificial Sequence: Synthetic polypeptide

SEQ ID NO: 240 - protein, 35 aa, synthetic construct; identical to SEQ ID NO: 2
  REGION 1..35: note = Description of Artificial Sequence: Synthetic polypeptide

SEQ ID NO: 241 - protein, 31 aa, synthetic construct; identical to SEQ ID NO: 67
  REGION 1..31: note = Description of Artificial Sequence: Synthetic polypeptide

SEQ ID NO: 242 - protein, 31 aa, synthetic construct
  REGION 1..31: note = Description of Artificial Sequence: Synthetic polypeptide
AEDQNDPYWARYADWLFTTPLLLLDLALLVG

SEQ ID NO: 243 - protein, 34 aa, synthetic construct; identical to SEQ ID NO: 31
  REGION 1..34: note = Description of Artificial Sequence: Synthetic polypeptide

SEQ ID NO: 244 - protein, 34 aa, synthetic construct
  REGION 1..34: note = Description of Artificial Sequence: Synthetic polypeptide
AEQNPIYFARYADWLFTTPLLLLDLALLVDADET

SEQ ID NO: 245 - protein, 34 aa, synthetic construct; identical to SEQ ID NO: 33
  REGION 1..34: note = Description of Artificial Sequence: Synthetic polypeptide

SEQ ID NO: 246 - protein, 36 aa, synthetic construct; identical to SEQ ID NO: 55
  REGION 1..36: note = Description of Artificial Sequence: Synthetic polypeptide

SEQ ID NO: 247 - protein, 34 aa, synthetic construct
  REGION 1..34: note = Description of Artificial Sequence: Synthetic polypeptide
AEDQNPIYWARYADWLFTTPLLLLDLALLVDCGT

SEQ ID NO: 248 - protein, 35 aa, synthetic construct
  REGION 1..35: note = Description of Artificial Sequence: Synthetic polypeptide
AEDQNDPIYWARYADWLFTTPLLLLELALLVECGT

SEQ ID NO: 249 - protein, 25 aa, synthetic construct
  REGION 1..25: note = Description of Artificial Sequence: Synthetic peptide
ACEEQNPWARYLEWLFPTETLLLEL

SEQ ID NO: 250 - protein, 35 aa, synthetic construct; identical to SEQ ID NO: 2
  REGION 1..35: note = Description of Artificial Sequence: Synthetic polypeptide

SEQ ID NO: 251 - protein, 32 aa, synthetic construct; identical to SEQ ID NO: 34
  REGION 1..32: note = Description of Artificial Sequence: Synthetic polypeptide

SEQ ID NO: 252 - protein, 32 aa, synthetic construct; identical to SEQ ID NO: 71
  REGION 1..32: note = Description of Artificial Sequence: Synthetic polypeptide

SEQ ID NO: 253 - protein, 35 aa, synthetic construct
  REGION 1..35: note = Description of Artificial Sequence: Synthetic polypeptide
AEQNPIYWARYADWLFTTPLLLLDLALLVDADEGC

SEQ ID NO: 254 - protein, 31 aa, synthetic construct
  REGION 1..31: note = Description of Artificial Sequence: Synthetic polypeptide
AEDQNPYWARYADWLFTTPLLLLDLALLVDC

SEQ ID NO: 255 - protein, 31 aa, synthetic construct
  REGION 1..31: note = Description of Artificial Sequence: Synthetic polypeptide
AEDQNPYWARYADWLFTTPLLLLELALLVEC

SEQ ID NO: 256 - protein, 36 aa, synthetic construct; identical to SEQ ID NO: 8
  REGION 1..36: note = Description of Artificial Sequence: Synthetic polypeptide

SEQ ID NO: 257 - protein, 32 aa, synthetic construct; identical to SEQ ID NO: 35
  REGION 1..32: note = Description of Artificial Sequence: Synthetic polypeptide

SEQ ID NO: 258 - protein, 30 aa, synthetic construct; identical to SEQ ID NO: 39
  REGION 1..30: note = Description of Artificial Sequence: Synthetic polypeptide

SEQ ID NO: 259 - protein, 27 aa, synthetic construct
  REGION 1..27: note = Description of Artificial Sequence: Synthetic peptide
ACDDQNPWRAYLDLLFPTDTLLLDLLW

SEQ ID NO: 260 - protein, 27 aa, synthetic construct
  REGION 1..27: note = Description of Artificial Sequence: Synthetic peptide
ACEEQNPWRAYLELLFPTETLLLELLW

SEQ ID NO: 261 - protein, 25 aa, synthetic construct
  REGION 1..25: note = Description of Artificial Sequence: Synthetic peptide
ACDDQNPWARYLDWLFPTDTLLLDL

SEQ ID NO: 262 - protein, 24 aa, synthetic construct
  REGION 1..24: note = Description of Artificial Sequence: Synthetic peptide
CDNNNPWRAYLDLLFPTDTLLLDW

SEQ ID NO: 263 - protein, 25 aa, synthetic construct
  REGION 1..25: note = Description of Artificial Sequence: Synthetic peptide
ACEEQNPWARYLEWLFPTETLLLEL

SEQ ID NO: 264 - protein, 24 aa, synthetic construct
  REGION 1..24: note = Description of Artificial Sequence: Synthetic peptide
CEEQQPWAQYLELLFPTETLLLEW

SEQ ID NO: 265 - protein, 24 aa, synthetic construct
  REGION 1..24: note = Description of Artificial Sequence: Synthetic peptide
CEEQQPWRAYLELLFPTETLLLEW

SEQ ID NO: 266 - protein, 24 aa, synthetic construct
  REGION 1..24: note = Description of Artificial Sequence: Synthetic peptide
ACEDQNPWARYADWLFPTTLLLLD

SEQ ID NO: 267 - protein, 24 aa, synthetic construct
  REGION 1..24: note = Description of Artificial Sequence: Synthetic peptide
ACEEQNPWARYAEWLFPTTLLLLE

SEQ ID NO: 268 - protein, 22 aa, synthetic construct
  REGION 1..22: note = Description of Artificial Sequence: Synthetic peptide
ACEDQNPWARYADLLFPTTLAW

SEQ ID NO: 269 - protein, 22 aa, synthetic construct
  REGION 1..22: note = Description of Artificial Sequence: Synthetic peptide
ACEEQNPWARYAELLFPTTLAW

SEQ ID NO: 270 - protein, 34 aa, synthetic construct; identical to SEQ ID NO: 41
  REGION 1..34: note = Description of Artificial Sequence: Synthetic polypeptide

SEQ ID NO: 271 - protein, 37 aa, synthetic construct
  REGION 1..37: note = Description of Artificial Sequence: Synthetic polypeptide
CDDDDDNPNYWARYANWLFTTPLLLLNGALLVEAEET

SEQ ID NO: 272 - protein, 37 aa, synthetic construct
  REGION 1..37: note = Description of Artificial Sequence: Synthetic polypeptide
CDDDDDNPNYWARYAPWLFTTPLLLLPGALLVEAEET

SEQ ID NO: 273 - skipped

SEQ ID NO: 274 - protein, 36 aa, synthetic construct; identical to SEQ ID NO: 55
  REGION 1..36: note = Description of Artificial Sequence: Synthetic polypeptide

SEQ ID NO: 275 - protein, 37 aa, synthetic construct
  REGION 1..37: note = Description of Artificial Sequence: Synthetic polypeptide
AKEQNPIYWARYADWLFTTPLLLLDLALLVDADEGTG

SEQ ID NO: 276 - protein, 36 aa, synthetic construct
  REGION 1..36: note = Description of Artificial Sequence: Synthetic polypeptide
ACEQNPIYWARYANWLFTTPLLLLNLALLVDADEGT

SEQ ID NO: 277 - protein, 36 aa, synthetic construct
  REGION 1..36: note = Description of Artificial Sequence: Synthetic polypeptide
DDDEDNPIYWARYADWLFTTPLLLLHGALLVDADET

SEQ ID NO: 278 - protein, 36 aa, synthetic construct; identical to SEQ ID NO: 277
  REGION 1..36: note = Description of Artificial Sequence: Synthetic polypeptide

SEQ ID NO: 279 - protein, 37 aa, synthetic construct
  REGION 1..37: note = Description of Artificial Sequence: Synthetic polypeptide
CDDDEDNPIYWARYAHWLFTTPLLLLHGALLVDADET

SEQ ID NO: 280 - protein, 37 aa, synthetic construct
  REGION 1..37: note = Description of Artificial Sequence: Synthetic polypeptide
DDDEDNPIYWARYAHWLFTTPLLLLHGALLVDADEGT

SEQ ID NO: 281 - protein, 37 aa, synthetic construct
  REGION 1..37: note = Description of Artificial Sequence: Synthetic polypeptide
DDDEDNPIYWARYAHWLFTTPLLLLHGALLVNADEGT

SEQ ID NO: 282 - protein, 37 aa, synthetic construct
  REGION 1..37: note = Description of Artificial Sequence: Synthetic polypeptide
DDDEDNPIYWARYAHWLFTTPLLLLHGALLVNANEGT

SEQ ID NO: 283 - protein, 32 aa, synthetic construct; identical to SEQ ID NO: 71
  REGION 1..32: note = Description of Artificial Sequence: Synthetic polypeptide

SEQ ID NO: 284 - protein, 31 aa, synthetic construct
  REGION 1..31: note = Description of Artificial Sequence: Synthetic polypeptide
AEDQNPYWARYADWLFTTPLLLLELALLVCG

SEQ ID NO: 285 - protein, 28 aa, synthetic construct
  REGION 1..28: note = Description of Artificial Sequence: Synthetic peptide
AKDDQNPWRAYLDLLFPTDTLLLDLLWC

SEQ ID NO: 286 - protein, 27 aa, synthetic construct
  REGION 1..27: note = Description of Artificial Sequence: Synthetic peptide
ACEEQNPWRAYLELLFPTETLLLELLW

SEQ ID NO: 287 - protein, 25 aa, synthetic construct
  REGION 1..25: note = Description of Artificial Sequence: Synthetic peptide
ACDDQNPWARYLDWLFPTDTLLLDL

SEQ ID NO: 288 - protein, 24 aa, synthetic construct
  REGION 1..24: note = Description of Artificial Sequence: Synthetic peptide
CDNNNPWRAYLDLLFPTDTLLLDW

SEQ ID NO: 289 - protein, 24 aa, synthetic construct
  REGION 1..24: note = Description of Artificial Sequence: Synthetic peptide
CEEQQPWAQYLELLFPTETLLLEW

SEQ ID NO: 290 - protein, 24 aa, synthetic construct
  REGION 1..24: note = Description of Artificial Sequence: Synthetic peptide
CEEQQPWRAYLELLFPTETLLLEW

SEQ ID NO: 291 - protein, 37 aa, synthetic construct; identical to SEQ ID NO: 271
  REGION 1..37: note = Description of Artificial Sequence: Synthetic polypeptide

SEQ ID NO: 292 - protein, 36 aa, synthetic construct
  REGION 1..36: note = Description of Artificial Sequence: Synthetic polypeptide
CDDDDDNPNYWARYAPWLFTTPLLLLPGALLVEAEE

SEQ ID NO: 293 - protein, 22 aa, synthetic construct
  REGION 1..22: note = Description of Artificial Sequence: Synthetic peptide
AEQNPIYFARYADLLFPTTLAW

SEQ ID NO: 294 - protein, 22 aa, synthetic construct
  REGION 1..22: note = Description of Artificial Sequence: Synthetic peptide
AEQNPIYWARYADLLFPTTLAF

SEQ ID NO: 295 - protein, 22 aa, synthetic construct
  REGION 1..22: note = Description of Artificial Sequence: Synthetic peptide
AEQNPIYWARYADLLFPTTLAW

SEQ ID NO: 296 - protein, 20 aa, synthetic construct
  REGION 1..20: note = Description of Artificial Sequence: Synthetic peptide
KEDQNPWARYADLLFPTTLW

SEQ ID NO: 297 - protein, 24 aa, synthetic construct
  REGION 1..24: note = Description of Artificial Sequence: Synthetic peptide
ACEEQNPQAEYAEWLFPTTLLLLE

SEQ ID NO: 298 - protein, 25 aa, synthetic construct
  REGION 1..25: note = Description of Artificial Sequence: Synthetic peptide
AAEEQNPWARYLEWLFPTETLLLEL

SEQ ID NO: 299 - protein, 25 aa, synthetic construct
  REGION 1..25: note = Description of Artificial Sequence: Synthetic peptide
AKEEQNPWARYLEWLFPTETLLLEL

SEQ ID NO: 300 - protein, 5 aa, synthetic construct
  REGION 1..5: note = Description of Artificial Sequence: Synthetic peptide
  MOD_RES 3: note = Any amino acid
WLXLL

SEQ ID NO: 301 - protein, 14 aa, synthetic construct
  REGION 1..14: note = Description of Artificial Sequence: Synthetic peptide
  MOD_RES 5: note = Any amino acid
AGWLXLLAGWLGLL

SEQ ID NO: 302 - protein, 5 aa, synthetic construct
  REGION 1..5: note = Description of Artificial Sequence: Synthetic peptide
  MOD_RES 3: note = Any amino acid
WIXLL

SEQ ID NO: 303 - protein, 5 aa, synthetic construct
  REGION 1..5: note = Description of Artificial Sequence: Synthetic peptide
  MOD_RES 3: note = Any amino acid
GGXGG

SEQ ID NO: 304 - protein, 6 aa, synthetic construct
  REGION 1..6: note = Description of Artificial Sequence: Synthetic 6xHis tag
HHHHHH

SEQ ID NO: 305 - protein, 4 aa, synthetic construct
  REGION 1..4: note = Description of Artificial Sequence: Synthetic peptide
AAEQ

SEQ ID NO: 306 - protein, 5 aa, synthetic construct
  REGION 1..5: note = Description of Artificial Sequence: Synthetic peptide
DDDED

SEQ ID NO: 307 - protein, 38 aa, unidentified
  REGION 1..38: note = Description of Unknown: Wild-type pH-sensitive membrane polypeptide
AAEQNPIYWARYADWLFTTPLLLLDLALLVDADEGTGG

SEQ ID NO: 308 - protein, 38 aa, synthetic construct
  REGION 1..38: note = Description of Artificial Sequence: Synthetic polypeptide
  MOD_RES 1: note = Ala or Asp
  MOD_RES 2: note = Ala, Asp or Cys
  MOD_RES 4: note = Gln or Asp
  MOD_RES 11: note = Arg or Gln
  MOD_RES 12: note = Tyr or Asp
  MOD_RES 13: note = Ala, Asp or Tyr
  MOD_RES 14: note = Asp, Asn, Glu, His, Lys, Ala or Trp
  MOD_RES 15: note = Trp or Asp
  MOD_RES 19: note = Thr or Asp
  MOD_RES 20: note = Pro, Gly or Ala
  MOD_RES 24: note = Leu or Asp
  MOD_RES 25: note = Asp, Leu, Asn, Glu, His, Lys or Ala
  MOD_RES 26: note = Leu, Asp or Gly
  MOD_RES 31: note = Asp or Asn
  MOD_RES 33: note = Asp or Asn
  MOD_RES 34: note = Glu or Gln
  MOD_RES 35: note = Gly or Cys
  MOD_RES 37: note = Gly or Cys
XXEXNPIYWAXXXXXLFTXXLLLXXXALLVXAXXXTXG

SEQ ID NO: 309 - protein, 42 aa, synthetic construct
  REGION 1..42: note = Description of Artificial Sequence: Synthetic polypeptide
  MOD_RES 1: note = May or may not be present
  MOD_RES 21: note = May or may not be present
  MOD_RES 29: note = May or may not be present
  MOD_RES 40: note = May or may not be present
DAAEQNPIYWARYADWLFTTLPLLLLDLLALLVDADEGTKGG

SEQ ID NO: 310 - protein, 38 aa, unidentified
  REGION 1..38: note = Description of Unknown: Wild-type pH-sensitive membrane polypeptide
GGEQNPIYWARYADWLFTTPLLLLDLALLVDADEGTGG

SEQ ID NO: 311 - protein, 38 aa, synthetic construct
  REGION 1..38: note = Description of Artificial Sequence: Synthetic polypeptide
  MOD_RES 1: note = Gly, Asp or Ala
  MOD_RES 2: note = Gly, Asp or Cys
  MOD_RES 4: note = Gln or Asp
  MOD_RES 11: note = Arg or Gln
  MOD_RES 12: note = Tyr or Asp
  MOD_RES 13: note = Ala, Asp or Tyr
  MOD_RES 14: note = Asp, Asn, Glu, His, Lys, Ala or Trp
  MOD_RES 15: note = Trp or Asp
  MOD_RES 19: note = Thr or Asp
  MOD_RES 20: note = Pro, Gly or Ala
  MOD_RES 24: note = Leu or Asp
  MOD_RES 25: note = Asp, Leu, Asn, Glu, His, Lys or Ala
  MOD_RES 26: note = Leu, Asp or Gly
  MOD_RES 31: note = Asp or Asn
  MOD_RES 33: note = Asp or Asn
  MOD_RES 34: note = Glu or Gln
  MOD_RES 35: note = Gly or Cys
XXEXNPIYWAXXXXXLFTXXLLLXXXALLVXAXXXTGG

SEQ ID NO: 312 - protein, 44 aa, synthetic construct
  REGION 1..44: note = Description of Artificial Sequence: Synthetic polypeptide
  MOD_RES 1: note = May or may not be present
  MOD_RES 7: note = May or may not be present
  MOD_RES 22: note = May or may not be present
  MOD_RES 30: note = May or may not be present
  MOD_RES 40: note = May or may not be present
  MOD_RES 42: note = Lys, Cys or absent
DGGEQNDPIYWARYADWLFTTLPLLLLDLLALLVDADEGCTXGG